European Patent Application EP 4 667 484 A1, published December 24, 2025. Title: HOMODIMERIC PROTEIN COMBINING HUMAN IL-1R1 WITH HUMAN IL-1RACP POLYPEPTIDE FRAGMENTS AND USE. Applicant: Zhejiang University. The sequence listing filed with the application follows.

SEQUENCE LISTING (20 sequences)

SEQ ID NO: 1 - DNA, 1710 bp, Homo sapiens
  source 1..1710: mol_type = genomic DNA
atgaaagtgttactcagacttatttgtttcatagctctactgatttcttctctggaggctgataaatgcaaggaacgtgaagaaaaaataattttagtgtcatctgcaaatgaaattgatgttcgtccctgtcctcttaacccaaatgaacacaaaggcactataacttggtataaagatgacagcaagacacctgtatctacagaacaagcctccaggattcatcaacacaaagagaaactttggtttgttcctgctaaggtggaggattcaggacattactattgcgtggtaagaaattcatcttactgcctcagaattaaaataagtgcaaaatttgtggagaatgagcctaacttatgttataatgcacaagccatatttaagcaggaactacccgttgcaggagacggaggacttgtgtgcccttatatggagttttttaaaaatgaaaataatgagttacctaaattacagtggtataaggattgcaaacctctacttcttgacaatatacactttagtggagtcaaagataggctcatcgtgatgaatgtggctgaaaagcatagagggaactatacttgtcatgcatcctacacatacttgggcaagcaatatcctattacccgggtaatagaatttattactctagaggaaaacaaacccacaaggcctgtgattgtgagcccagctaatgagacaatggaagtagacttgggatcccagatacaattgatctgtaatgtcaccggccagttgagtgacattgcttactggaagtggaatgggtcagtaattgatgaagatgacccagtgctaggggaagactattacagtgtggaaaatcctgcaaacaaaagaaggagtaccctcatcacagtgcttaatatatcggaaattgaaagtagattttataaacatccatttacctgttttgccaagaatacacatggtatagatgcagcatatatccagttaatatatccagtcactaatttccagaagcacatgattggtatatgtgtcacgttgacagtcataattgtgtgttctgttttcatctataaaatcttcaagattgacattgtgctttggtacagggattcctgctatgattttctcccaataaaagcttcagatggaaagacctatgacgcatatatactgtatccaaagactgttggggaagggtctacctctgactgtgatatttttgtgtttaaagtcttgcctgaggtcttggaaaaacagtgtggatataagctgttcatttatggaagggatgactacgttggggaagacattgttgaggtcattaatgaaaacgtaaagaaaagcagaagactgattatcattttagtcagagaaacatcaggcttcagctggctgggtggttcatctgaagagcaaatagccatgtataatgctcttgttcaggatggaattaaagttgtcctgcttgagctggagaaaatccaagactatgagaaaatgccagaatcgattaaattcattaagcagaaacatggggctatccgctggtcaggggactttacacagggaccacagtctgcaaagacaaggttctggaagaatgtcaggtaccacatgccagtccagcgacggtcaccttcatctaaacaccagttactgtcaccagccactaaggagaaactgcaaagagaggctcacgtgcctctcgggtag

SEQ ID NO: 2 - DNA, 1710 bp, synthetic construct
  source 1..1710: mol_type = other DNA
atgaaagtgttactcagacttatttgtttcatagctctactgatttcttctctggaggctgataaatgcaaggaacgtgaagaaaaaataattttagtgtcatctgcaaatgaaattgatgttcgtccctgtcctcttaacccaaatgaacacaaaggcactataacttggtataaagatgacagcaagacacctgtatctacagaacaagcctccaggattcatcaacacaaagagaaactttggtttgttcctgctaaggtggaggattcaggacattactattgcgtggtaagaaattcatcttactgcctcagaattaaaataagtgcaaaatttgtggagaatgagcctaacttatgttataatgcacaagccatatttaagcaggacctacccgttgcaggagacggaggacttgtgtgcccttatatggagttttttaaaaatgaaaataatgagttacctaaattacagtggtataaggattgcaaacctctacttcttgacaatatacactttagtggagtcaaagataggctcatcgtgatgaatgtggctgaaaagcatagagggaactatacttgtcatgcatcctacacatacttgggcaagcaatatcctattacccgggtaatagaatttattactctagaggaaaacaaacccacaaggcctgtgattgtgagcccagctaatgagacaatggaagtagacttgggatcccagatacaattgatctgtaatgtcaccggccagttgagtgacattgcttactggaagtggaatgggtcagtaattgatgaagatgacccagtgctaggggaagactattacagtgtggaaaatcctgcaaacaaaagaaggagtaccctcatcacagtgcttaatatatcggaaattgaaagtagattttataaacatccatttacctgttttgccaagaatacacatggtatagatgcagcatatatccagttaatatatccagtcactaatttccagaagcacatgattggtatatgtgtcacgttgacagtcataattgtgtgttctgttttcatctataaaatcttcaagattgacattgtgctttggtacagggattcctgctatgattttctcccaataaaagcttcagatggaaagacctatgacgcatatatactgtatccaaagactgttggggaagggtctacctctgactgtgatatttttgtgtttaaagtcttgcctgaggtcttggaaaaacagtgtggatataagctgttcatttatggaagggatgactacgttggggaagacattgttgaggtcattaatgaaaacgtaaagaaaagcagaagactgattatcattttagtcagagaaacatcaggcttcagctggctgggtggttcatctgaagagcaaatagccatgtataatgctcttgttcaggatggaattaaagttgtcctgcttgagctggagaaaatccaagactatgagaaaatgccagaatcgattaaattcattaagcagaaacatggggctatccgctggtcaggggactttacacagggaccacagtctgcaaagacaaggttctggaagaatgtcaggtaccacatgccagtccagcgacggtcaccttcatctaaacaccagttactgtcaccagccactaaggagaaactgcaaagagaggctcacgtgcctctcgggtag

SEQ ID NO: 3 - protein, 569 aa, Homo sapiens
MKVLLRLICFIALLISSLEADKCKEREEKIILVSSANEIDVRPCPLNPNEHKGTITWYKDDSKTPVSTEQASRIHQHKEKLWFVPAKVEDSGHYYCVVRNSSYCLRIKISAKFVENEPNLCYNAQAIFKQELPVAGDGGLVCPYMEFFKNENNELPKLQWYKDCKPLLLDNIHFSGVKDRLIVMNVAEKHRGNYTCHASYTYLGKQYPITRVIEFITLEENKPTRPVIVSPANETMEVDLGSQIQLICNVTGQLSDIAYWKWNGSVIDEDDPVLGEDYYSVENPANKRRSTLITVLNISEIESRFYKHPFTCFAKNTHGIDAAYIQLIYPVTNFQKHMIGICVTLTVIIVCSVFIYKIFKIDIVLWYRDSCYDFLPIKASDGKTYDAYILYPKTVGEGSTSDCDIFVFKVLPEVLEKQCGYKLFIYGRDDYVGEDIVEVINENVKKSRRLIIILVRETSGFSWLGGSSEEQIAMYNALVQDGIKVVLLELEKIQDYEKMPESIKFIKQKHGAIRWSGDFTQGPQSAKTRFWKNVRYHMPVQRRSPSSKHQLLSPATKEKLQREAHVPLG

SEQ ID NO: 4 - protein, 569 aa, synthetic construct
MKVLLRLICFIALLISSLEADKCKEREEKIILVSSANEIDVRPCPLNPNEHKGTITWYKDDSKTPVSTEQASRIHQHKEKLWFVPAKVEDSGHYYCVVRNSSYCLRIKISAKFVENEPNLCYNAQAIFKQDLPVAGDGGLVCPYMEFFKNENNELPKLQWYKDCKPLLLDNIHFSGVKDRLIVMNVAEKHRGNYTCHASYTYLGKQYPITRVIEFITLEENKPTRPVIVSPANETMEVDLGSQIQLICNVTGQLSDIAYWKWNGSVIDEDDPVLGEDYYSVENPANKRRSTLITVLNISEIESRFYKHPFTCFAKNTHGIDAAYIQLIYPVTNFQKHMIGICVTLTVIIVCSVFIYKIFKIDIVLWYRDSCYDFLPIKASDGKTYDAYILYPKTVGEGSTSDCDIFVFKVLPEVLEKQCGYKLFIYGRDDYVGEDIVEVINENVKKSRRLIIILVRETSGFSWLGGSSEEQIAMYNALVQDGIKVVLLELEKIQDYEKMPESIKFIKQKHGAIRWSGDFTQGPQSAKTRFWKNVRYHMPVQRRSPSSKHQLLSPATKEKLQREAHVPLG

SEQ ID NO: 5 - protein, 339 aa, Homo sapiens
SERCDDWGLDTMRQIQVFEDEPARIKCPLFEHFLKFNYSTAHSAGLTLIWYWTRQDRDLEEPINFRLPENRISKEKDVLWFRPTLLNDTGNYTCMLRNTTYCSKVAFPLEVVQKDSCFNSPMKLPVHKLYIEYGIQRITCPNVDGYFPSSVKPTITWYMGCYKIQNFNNVIPEGMNLSFLIALISNNGNYTCVVTYPENGRTFHLTRTLTVKVVGSPKNAVPPVIHSPNDHVVYEKEPGEELLIPCTVYFSFLMDSRNEVWWTIDGKKPDDITIDVTINESISHSRTEDETRTQILSIKKVTSEDLKRSYVCHARSAKGEVAKAAKVKQKVPAPRYTVE

SEQ ID NO: 6 - protein, 332 aa, Homo sapiens
MKVLLRLICFIALLISSLEADKCKEREEKIILVSSANEIDVRPCPLNPNEHKGTITWYKDDSKTPVSTEQASRIHQHKEKLWFVPAKVEDSGHYYCVVRNSSYCLRIKISAKFVENEPNLCYNAQAIFKQELPVAGDGGLVCPYMEFFKNENNELPKLQWYKDCKPLLLDNIHFSGVKDRLIVMNVAEKHRGNYTCHASYTYLGKQYPITRVIEFITLEENKPTRPVIVSPANETMEVDLGSQIQLICNVTGQLSDIAYWKWNGSVIDEDDPVLGEDYYSVENPANKRRSTLITVLNISEIESRFYKHPFTCFAKNTHGIDAAYIQLIYPVT

SEQ ID NO: 7 - protein, 332 aa, synthetic construct
MKVLLRLICFIALLISSLEADKCKEREEKIILVSSANEIDVRPCPLNPNEHKGTITWYKDDSKTPVSTEQASRIHQHKEKLWFVPAKVEDSGHYYCVVRNSSYCLRIKISAKFVENEPNLCYNAQAIFKQDLPVAGDGGLVCPYMEFFKNENNELPKLQWYKDCKPLLLDNIHFSGVKDRLIVMNVAEKHRGNYTCHASYTYLGKQYPITRVIEFITLEENKPTRPVIVSPANETMEVDLGSQIQLICNVTGQLSDIAYWKWNGSVIDEDDPVLGEDYYSVENPANKRRSTLITVLNISEIESRFYKHPFTCFAKNTHGIDAAYIQLIYPVT

SEQ ID NO: 8 - protein, 238 aa, Homo sapiens
ADDDDKEPKSSDKTHTCPPCPAPELLGGPSVFLFPPKPKDTLMISRTPEVTCVVVDVSHEDPEVKFNWYVDGVEVHNAKTKPREEQYNSTYRVVSVLTVLHQDWLNGKEYKCKVSNKALPAPIEKTISKAKGQPREPQVYTLPPSRDELTKNQVSLTCLVKGFYPSDIAVEWESNGQPENNYKTTPPVLDSDGSFFLYSKLTVDKSRWQQGNVFSCSVMHEALHNHYTQKSLSLSPGK

SEQ ID NO: 9 - protein, 900 aa, synthetic construct
MGLLWYLMSLSFYGILQSHASERCDDWGLDTMRQIQVFEDEPARIKCPLFEHFLKFNYSTAHSAGLTLIWYWTRQDRDLEEPINFRLPENRISKEKDVLWFRPTLLNDTGNYTCMLRNTTYCSKVAFPLEVVQKDSCFNSPMKLPVHKLYIEYGIQRITCPNVDGYFPSSVKPTITWYMGCYKIQNFNNVIPEGMNLSFLIALISNNGNYTCVVTYPENGRTFHLTRTLTVKVVGSPKNAVPPVIHSPNDHVVYEKEPGEELLIPCTVYFSFLMDSRNEVWWTIDGKKPDDITIDVTINESISHSRTEDETRTQILSIKKVTSEDLKRSYVCHARSAKGEVAKAAKVKQKVPAPRYTVEKCKEREEKIILVSSANEIDVRPCPLNPNEHKGTITWYKDDSKTPVSTEQASRIHQHKEKLWFVPAKVEDSGHYYCVVRNSSYCLRIKISAKFVENEPNLCYNAQAIFKQELPVAGDGGLVCPYMEFFKNENNELPKLQWYKDCKPLLLDNIHFSGVKDRLIVMNVAEKHRGNYTCHASYTYLGKQYPITRVIEFITLEENKPTRPVIVSPANETMEVDLGSQIQLICNVTGQLSDIAYWKWNGSVIDEDDPVLGEDYYSVENPANKRRSTLITVLNISEIESRFYKHPFTCFAKNTHGIDAAYIQLIYPVTNSGDKTHTCPPCPAPELLGGPSVFLFPPKPKDTLMISRTPEVTCVVVDVSHEDPEVKFNWYVDGVEVHNAKTKPREEQYNSTYRVVSVLTVLHQDWLNGKEYKCKVSNKALPAPIEKTISKAKGQPREPQVYTLPPSRDELTKNQVSLTCLVKGFYPSDIAVEWESNGQPENNYKTTPPVLDSDGSFFLYSKLTVDKSRWQQGNVFSCSVMHEALHNHYTQKSLSLSPGK

SEQ ID NO: 10 - protein, 900 aa, synthetic construct
MGLLWYLMSLSFYGILQSHASERCDDWGLDTMRQIQVFEDEPARIKCPLFEHFLKFNYSTAHSAGLTLIWYWTRQDRDLEEPINFRLPENRISKEKDVLWFRPTLLNDTGNYTCMLRNTTYCSKVAFPLEVVQKDSCFNSPMKLPVHKLYIEYGIQRITCPNVDGYFPSSVKPTITWYMGCYKIQNFNNVIPEGMNLSFLIALISNNGNYTCVVTYPENGRTFHLTRTLTVKVVGSPKNAVPPVIHSPNDHVVYEKEPGEELLIPCTVYFSFLMDSRNEVWWTIDGKKPDDITIDVTINESISHSRTEDETRTQILSIKKVTSEDLKRSYVCHARSAKGEVAKAAKVKQKVPAPRYTVEKCKEREEKIILVSSANEIDVRPCPLNPNEHKGTITWYKDDSKTPVSTEQASRIHQHKEKLWFVPAKVEDSGHYYCVVRNSSYCLRIKISAKFVENEPNLCYNAQAIFKQDLPVAGDGGLVCPYMEFFKNENNELPKLQWYKDCKPLLLDNIHFSGVKDRLIVMNVAEKHRGNYTCHASYTYLGKQYPITRVIEFITLEENKPTRPVIVSPANETMEVDLGSQIQLICNVTGQLSDIAYWKWNGSVIDEDDPVLGEDYYSVENPANKRRSTLITVLNISEIESRFYKHPFTCFAKNTHGIDAAYIQLIYPVTNSGDKTHTCPPCPAPELLGGPSVFLFPPKPKDTLMISRTPEVTCVVVDVSHEDPEVKFNWYVDGVEVHNAKTKPREEQYNSTYRVVSVLTVLHQDWLNGKEYKCKVSNKALPAPIEKTISKAKGQPREPQVYTLPPSRDELTKNQVSLTCLVKGFYPSDIAVEWESNGQPENNYKTTPPVLDSDGSFFLYSKLTVDKSRWQQGNVFSCSVMHEALHNHYTQKSLSLSPGK

SEQ ID NO: 11 - DNA, 2703 bp, synthetic construct
  source 1..2703: mol_type = other DNA
atggtgcttctgtggtgtgtagtgagtctctacttttatggaatcctgcaaagtgatgcctcagaacgctgcgatgactggggactagacaccatgaggcaaatccaagtgtttgaagatgagccagctcgcatcaagtgcccactctttgaacacttcttgaaattcaactacagcacagcccattcagctggccttactctgatctggtattggactaggcaggaccgggaccttgaggagccaattaacttccgcctccccgagaaccgcattagtaaggagaaagatgtgctgtggttccggcccactctcctcaatgacactggcaactatacctgcatgttaaggaacactacatattgcagcaaagttgcatttcccttggaagttgttcaaaaagacagctgtttcaattcccccatgaaactcccagtgcataaactgtatatagaatatggcattcagaggatcacttgtccaaatgtagatggatattttccttccagtgtcaaaccgactatcacttggtatatgggctgttataaaatacagaattttaataatgtaatacccgaaggtatgaacttgagtttcctcattgccttaatttcaaataatggaaattacacatgtgttgttacatatccagaaaatggacgtacgtttcatctcaccaggactctgactgtaaaggtagtaggctctccaaaaaatgcagtgccccctgtgatccattcacctaatgatcatgtggtctatgagaaagaaccaggagaggagctactcattccctgtacggtctattttagttttctgatggattctcgcaatgaggtttggtggaccattgatggaaaaaaacctgatgacatcactattgatgtcaccattaacgaaagtataagtcatagtagaacagaagatgaaacaagaactcagattttgagcatcaagaaagttacctctgaggatctcaagcgcagctatgtctgtcatgctagaagtgccaaaggcgaagttgccaaagcagccaaggtgaagcagaaagtgccagctccaagatacacagtggaaaaatgcaaggaacgtgaagaaaaaataattttagtgtcatctgcaaatgaaattgatgttcgtccctgtcctcttaacccaaatgaacacaaaggcactataacttggtataaagatgacagcaagacacctgtatctacagaacaagcctccaggattcatcaacacaaagagaaactttggtttgttcctgctaaggtggaggattcaggacattactattgcgtggtaagaaattcatcttactgcctcagaattaaaataagtgcaaaatttgtggagaatgagcctaacttatgttataatgcacaagccatatttaagcaggaactacccgttgcaggagacggaggacttgtgtgcccttatatggagttttttaaaaatgaaaataatgagttacctaaattacagtggtataaggattgcaaacctctacttcttgacaatatacactttagtggagtcaaagataggctcatcgtgatgaatgtggctgaaaagcatagagggaactatacttgtcatgcatcctacacatacttgggcaagcaatatcctattacccgggtaatagaatttattactctagaggaaaacaaacccacaaggcctgtgattgtgagcccagctaatgagacaatggaagtagacttgggatcccagatacaattgatctgtaatgtcaccggccagttgagtgacattgcttactggaagtggaatgggtcagtaattgatgaagatgacccagtgctaggggaagactattacagtgtggaaaatcctgcaaacaaaagaaggagtaccctcatcacagtgcttaatatatcggaaattgaaagtagattttataaacatccatttacctgttttgccaagaatacacatggtatagatgcagcatatatccagttaatatatccagtcactaattctggtgacaaaactcacacatgcccaccgtgcccagcacctgaactcctggggggaccgtcagtcttcctcttccccccaaaacccaaggacaccctcatgatctcccggacccctgaggtcacgtgcgtggtggtggacgtgagccacgaagaccccgaggtcaagttcaactggtacgtggacggcgtggaggtgcataatgccaagacaaagccgcgggaggagcagtacaacagcacgtaccgtgtggtcagcgtcctcaccgtcctgcaccaggactggctgaatggcaaggagtacaagtgcaaggtctccaacaaagccctcccagcccccatcgagaaaaccatctccaaagccaaagggcagccccgagaaccacaggtgtacaccctgcccccatcccgggatgagctgaccaagaaccaggtcagcctgacctgcctggtcaaaggcttctatcccagcgacatcgccgtggagtgggagagcaatgggcagccggagaacaactacaagaccacgcctcccgtgctggactccgacggctccttcttcctctacagcaagctcaccgtggacaagagcaggtggcagcaggggaacgtcttctcatgctccgtgatgcatgaggctctgcacaaccactacacgcagaagagcctctccctgtctccgggtaaatga

SEQ ID NO: 12 - DNA, 2703 bp, synthetic construct
  source 1..2703: mol_type = other DNA
atggtgcttctgtggtgtgtagtgagtctctacttttatggaatcctgcaaagtgatgcctcagaacgctgcgatgactggggactagacaccatgaggcaaatccaagtgtttgaagatgagccagctcgcatcaagtgcccactctttgaacacttcttgaaattcaactacagcacagcccattcagctggccttactctgatctggtattggactaggcaggaccgggaccttgaggagccaattaacttccgcctccccgagaaccgcattagtaaggagaaagatgtgctgtggttccggcccactctcctcaatgacactggcaactatacctgcatgttaaggaacactacatattgcagcaaagttgcatttcccttggaagttgttcaaaaagacagctgtttcaattcccccatgaaactcccagtgcataaactgtatatagaatatggcattcagaggatcacttgtccaaatgtagatggatattttccttccagtgtcaaaccgactatcacttggtatatgggctgttataaaatacagaattttaataatgtaatacccgaaggtatgaacttgagtttcctcattgccttaatttcaaataatggaaattacacatgtgttgttacatatccagaaaatggacgtacgtttcatctcaccaggactctgactgtaaaggtagtaggctctccaaaaaatgcagtgccccctgtgatccattcacctaatgatcatgtggtctatgagaaagaaccaggagaggagctactcattccctgtacggtctattttagttttctgatggattctcgcaatgaggtttggtggaccattgatggaaaaaaacctgatgacatcactattgatgtcaccattaacgaaagtataagtcatagtagaacagaagatgaaacaagaactcagattttgagcatcaagaaagttacctctgaggatctcaagcgcagctatgtctgtcatgctagaagtgccaaaggcgaagttgccaaagcagccaaggtgaagcagaaagtgccagctccaagatacacagtggaaaaatgcaaggaacgtgaagaaaaaataattttagtgtcatctgcaaatgaaattgatgttcgtccctgtcctcttaacccaaatgaacacaaaggcactataacttggtataaagatgacagcaagacacctgtatctacagaacaagcctccaggattcatcaacacaaagagaaactttggtttgttcctgctaaggtggaggattcaggacattactattgcgtggtaagaaattcatcttactgcctcagaattaaaataagtgcaaaatttgtggagaatgagcctaacttatgttataatgcacaagccatatttaagcaggacctacccgttgcaggagacggaggacttgtgtgcccttatatggagttttttaaaaatgaaaataatgagttacctaaattacagtggtataaggattgcaaacctctacttcttgacaatatacactttagtggagtcaaagataggctcatcgtgatgaatgtggctgaaaagcatagagggaactatacttgtcatgcatcctacacatacttgggcaagcaatatcctattacccgggtaatagaatttattactctagaggaaaacaaacccacaaggcctgtgattgtgagcccagctaatgagacaatggaagtagacttgggatcccagatacaattgatctgtaatgtcaccggccagttgagtgacattgcttactggaagtggaatgggtcagtaattgatgaagatgacccagtgctaggggaagactattacagtgtggaaaatcctgcaaacaaaagaaggagtaccctcatcacagtgcttaatatatcggaaattgaaagtagattttataaacatccatttacctgttttgccaagaatacacatggtatagatgcagcatatatccagttaatatatccagtcactaattctggtgacaaaactcacacatgcccaccgtgcccagcacctgaactcctggggggaccgtcagtcttcctcttccccccaaaacccaaggacaccctcatgatctcccggacccctgaggtcacgtgcgtggtggtggacgtgagccacgaagaccccgaggtcaagttcaactggtacgtggacggcgtggaggtgcataatgccaagacaaagccgcgggaggagcagtacaacagcacgtaccgtgtggtcagcgtcctcaccgtcctgcaccaggactggctgaatggcaaggagtacaagtgcaaggtctccaacaaagccctcccagcccccatcgagaaaaccatctccaaagccaaagggcagccccgagaaccacaggtgtacaccctgcccccatcccgggatgagctgaccaagaaccaggtcagcctgacctgcctggtcaaaggcttctatcccagcgacatcgccgtggagtgggagagcaatgggcagccggagaacaactacaagaccacgcctcccgtgctggactccgacggctccttcttcctctacagcaagctcaccgtggacaagagcaggtggcagcaggggaacgtcttctcatgctccgtgatgcatgaggctctgcacaaccactacacgcagaagagcctctccctgtctccgggtaaatga

SEQ ID NO: 13 - protein, 339 aa, Mus musculus
SERCDDWGLDTMRQIQVFEDEPARIKCPLFEHFLKYNYSTAHSSGLTLIWYWTRQDRDLEEPINFRLPENRISKEKDVLWFRPTLLNDTGNYTCMLRNTTYCSKVAFPLEVVQKDSCFNSAMRFPVHKMYIEHGIHKITCPNVDGYFPSSVKPSVTWYKGCTEIVDFHNVLPEGMNLSFFIPLVSNNGNYTCVVTYPENGRLFHLTRTVTVKVVGSPKDALPPQIYSPNDRVVYEKEPGEELVIPCKVYFSFIMDSHNEVWWTIDGKKPDDVTVDITINESVSYSSTEDETRTQILSIKKVTPEDLRRNYVCHARNTKGEAEQAAKVKQKVIPPRYTVE

SEQ ID NO: 14 - protein, 313 aa, synthetic construct
VCTEYPNQIVLFLSVNEIDIRKCPLTPNKMHGDTIIWYKNDSKTPISADRDSRIHQQNEHLWFVPAKVEDSGYYYCIVRNSTYCLKTKVTVTVLENDPGLCYSTQATFPQELHIAGDGSLVCPYVSYFKDENNELPEVQWYKNCKPLLLDNVSFFGVKDKLLVRNVAEEHRGDYICRMSYTFRGKQYPVTRVIQFITIDENKRDRPVILSPRNETIEADPGSMIQLICNVTGQFSDLVYWKWNGSEIEWNDPFLAEDYQFVEHPSTKRKYTLITTLNISEVKSQFYRYPFICVVKNTNIFESAHVQLIYPVPD

SEQ ID NO: 15 - protein, 313 aa, synthetic construct
VCTEYPNQIVLFLSVNEIDIRKCPLTPNKMHGDTIIWYKNDSKTPISADRDSRIHQQNEHLWFVPAKVEDSGYYYCIVRNSTYCLKTKVTVTVLENDPGLCYSTQATFPQDLHIAGDGSLVCPYVSYFKDENNELPEVQWYKNCKPLLLDNVSFFGVKDKLLVRNVAEEHRGDYICRMSYTFRGKQYPVTRVIQFITIDENKRDRPVILSPRNETIEADPGSMIQLICNVTGQFSDLVYWKWNGSEIEWNDPFLAEDYQFVEHPSTKRKYTLITTLNISEVKSQFYRYPFICVVKNTNIFESAHVQLIYPVPD

SEQ ID NO: 16 - protein, 228 aa, Mus musculus
DVPRDSGCKPCICTVPEVSSVFIFPPKPKDVLTITLTPKVTCVVVDISKDDPEVQFSWFVDDVEVHTAQTQPREEQFNSTFRSVSELPIMHQDWLNGKEFKCRVNSAAFPAPIEKTISKTKGRPKAPQVYTIPPPKEQMAKDKVSLTCMITDFFPEDITVEWQWNGQPAENYKNTQPIMDTDGSYFVYSKLNVQKSNWEAGNTFTCSVLHEGLHNHHTEKSLSHSPGK

SEQ ID NO: 17 - protein, 903 aa, synthetic construct
MGLLWYLMSLSFYGILQSHASERCDDWGLDTMRQIQVFEDEPARIKCPLFEHFLKYNYSTAHSSGLTLIWYWTRQDRDLEEPINFRLPENRISKEKDVLWFRPTLLNDTGNYTCMLRNTTYCSKVAFPLEVVQKDSCFNSAMRFPVHKMYIEHGIHKITCPNVDGYFPSSVKPSVTWYKGCTEIVDFHNVLPEGMNLSFFIPLVSNNGNYTCVVTYPENGRLFHLTRTVTVKVVGSPKDALPPQIYSPNDRVVYEKEPGEELVIPCKVYFSFIMDSHNEVWWTIDGKKPDDVTVDITINESVSYSSTEDETRTQILSIKKVTPEDLRRNYVCHARNTKGEAEQAAKVKQKVIPPRYTVEVCTEYPNQIVLFLSVNEIDIRKCPLTPNKMHGDTIIWYKNDSKTPISADRDSRIHQQNEHLWFVPAKVEDSGYYYCIVRNSTYCLKTKVTVTVLENDPGLCYSTQATFPQELHIAGDGSLVCPYVSYFKDENNELPEVQWYKNCKPLLLDNVSFFGVKDKLLVRNVAEEHRGDYICRMSYTFRGKQYPVTRVIQFITIDENKRDRPVILSPRNETIEADPGSMIQLICNVTGQFSDLVYWKWNGSEIEWNDPFLAEDYQFVEHPSTKRKYTLITTLNISEVKSQFYRYPFICVVKNTNIFESAHVQLIYPVPDNSGDVPRDSGCKPCICTVPEVSSVFIFPPKPKDVLTITLTPKVTCVVVDISKDDPEVQFSWFVDDVEVHTAQTQPREEQFNSTFRSVSELPIMHQDWLNGKEFKCRVNSAAFPAPIEKTISKTKGRPKAPQVYTIPPPKEQMAKDKVSLTCMITDFFPEDITVEWQWNGQPAENYKNTQPIMDTDGSYFVYSKLNVQKSNWEAGNTFTCSVLHEGLHNHHTEKSLSHSPGK

SEQ ID NO: 18 - protein, 903 aa, synthetic construct
MGLLWYLMSLSFYGILQSHASERCDDWGLDTMRQIQVFEDEPARIKCPLFEHFLKYNYSTAHSSGLTLIWYWTRQDRDLEEPINFRLPENRISKEKDVLWFRPTLLNDTGNYTCMLRNTTYCSKVAFPLEVVQKDSCFNSAMRFPVHKMYIEHGIHKITCPNVDGYFPSSVKPSVTWYKGCTEIVDFHNVLPEGMNLSFFIPLVSNNGNYTCVVTYPENGRLFHLTRTVTVKVVGSPKDALPPQIYSPNDRVVYEKEPGEELVIPCKVYFSFIMDSHNEVWWTIDGKKPDDVTVDITINESVSYSSTEDETRTQILSIKKVTPEDLRRNYVCHARNTKGEAEQAAKVKQKVIPPRYTVEVCTEYPNQIVLFLSVNEIDIRKCPLTPNKMHGDTIIWYKNDSKTPISADRDSRIHQQNEHLWFVPAKVEDSGYYYCIVRNSTYCLKTKVTVTVLENDPGLCYSTQATFPQDLHIAGDGSLVCPYVSYFKDENNELPEVQWYKNCKPLLLDNVSFFGVKDKLLVRNVAEEHRGDYICRMSYTFRGKQYPVTRVIQFITIDENKRDRPVILSPRNETIEADPGSMIQLICNVTGQFSDLVYWKWNGSEIEWNDPFLAEDYQFVEHPSTKRKYTLITTLNISEVKSQFYRYPFICVVKNTNIFESAHVQLIYPVPDNSGDVPRDSGCKPCICTVPEVSSVFIFPPKPKDVLTITLTPKVTCVVVDISKDDPEVQFSWFVDDVEVHTAQTQPREEQFNSTFRSVSELPIMHQDWLNGKEFKCRVNSAAFPAPIEKTISKTKGRPKAPQVYTIPPPKEQMAKDKVSLTCMITDFFPEDITVEWQWNGQPAENYKNTQPIMDTDGSYFVYSKLNVQKSNWEAGNTFTCSVLHEGLHNHHTEKSLSHSPGK

SEQ ID NO: 19 - DNA, 2016 bp, synthetic construct
  source 1..2016: mol_type = other DNA
atgggacttctgtggtatttgatgagtctgtccttctatgggatcctgcagagtcatgcttcggagcgctgtgatgactggggactagataccatgcgacaaatccaagtgtttgaagatgagccggctcgaatcaagtgccccctctttgaacacttcctgaagtacaactacagcactgcccattcctctggccttaccctgatctggtactggaccaggcaagaccgggacctggaggagcccattaacttccgcctcccagagaatcgcatcagtaaggagaaagatgtgctctggttccggcccaccctcctcaatgacacgggcaattacacctgcatgttgaggaacacaacttactgcagcaaagttgcatttcccctggaagttgttcagaaggacagctgtttcaattctgccatgagattcccagtgcacaagatgtatattgaacatggcattcataagatcacatgtccaaatgtagacggatactttccttccagtgtcaaaccatcggtcacttggtataagggttgtactgaaatagtggactttcataatgtactacccgagggcatgaacttgagctttttcatccccttggtttcaaataacggaaattacacatgtgtggttacatatcctgaaaacggacgtctctttcacctcaccaggactgtgactgtaaaggtggtgggctcaccaaaggatgcattgccaccccagatctattctccaaatgaccgtgttgtctatgagaaagaaccaggagaggaactggttattccctgcaaagtctatttcagtttcattatggactcccacaatgaggtctggtggaccattgatggaaagaagcctgatgacgtcacagtcgacatcactattaatgaaagtgtaagttattcttcaacggaagatgaaacaaggactcagattttgagcatcaagaaagtcaccccggaggatctcaggcgcaactatgtctgtcatgctcgaaataccaaaggggaagctgagcaggctgccaaggtgaaacagaaagtcataccaccaaggtacacagtagaagtatgtacagaatatccaaatcagatcgttttgtttttatctgtaaatgaaattgatattcgcaagtgtcctcttactccaaataaaatgcacggcgacaccataatttggtacaagaatgacagcaagacccccatatcagcggaccgggactccaggattcatcagcagaatgaacatctttggtttgtacctgccaaggtggaggactcaggatattactattgtatagtaagaaactcaacttactgcctcaaaactaaagtaaccgtaactgtgttagagaatgaccctggcttgtgttacagcacacaggccaccttcccacaggagctccacattgccggggatggaagtcttgtgtgcccttatgtgagttattttaaagatgaaaataatgagttacccgaggtccagtggtataagaactgtaaacctctgcttcttgacaacgtgagcttcttcggagtaaaagataaactgttggtgaggaatgtggctgaagagcacagaggggactatatatgccgtatgtcctatacgttccgggggaagcaatatccggtcacacgagtaatacaatttatcacaatagatgaaaacaagagggacagacctgttatcctgagccctcggaatgagacgatcgaagctgacccaggatcaatgatacaactgatctgcaacgtcacgggccagttctcagaccttgtctactggaagtggaatggatcagaaattgaatggaatgatccatttctagctgaagactatcaatttgtggaacatccttcaaccaaaagaaaatacacactcattacaacacttaacatttcagaagttaaaagccagttttatcgctatccgtttatctgtgttgttaagaacacaaatatttttgagtcggcgcatgtgcagttaatatacccagtccctgac

SEQ ID NO: 20 - DNA, 2727 bp, synthetic construct
  source 1..2727: mol_type = other DNA
atgggacttctgtggtatttgatgagtctgtccttctatgggatcctgcagagtcatgcttcggagcgctgtgatgactggggactagataccatgcgacaaatccaagtgtttgaagatgagccggctcgaatcaagtgccccctctttgaacacttcctgaagtacaactacagcactgcccattcctctggccttaccctgatctggtactggaccaggcaagaccgggacctggaggagcccattaacttccgcctcccagagaatcgcatcagtaaggagaaagatgtgctctggttccggcccaccctcctcaatgacacgggcaattacacctgcatgttgaggaacacaacttactgcagcaaagttgcatttcccctggaagttgttcagaaggacagctgtttcaattctgccatgagattcccagtgcacaagatgtatattgaacatggcattcataagatcacatgtccaaatgtagacggatactttccttccagtgtcaaaccatcggtcacttggtataagggttgtactgaaatagtggactttcataatgtactacccgagggcatgaacttgagctttttcatccccttggtttcaaataacggaaattacacatgtgtggttacatatcctgaaaacggacgtctctttcacctcaccaggactgtgactgtaaaggtggtgggctcaccaaaggatgcattgccaccccagatctattctccaaatgaccgtgttgtctatgagaaagaaccaggagaggaactggttattccctgcaaagtctatttcagtttcattatggactcccacaatgaggtctggtggaccattgatggaaagaagcctgatgacgtcacagtcgacatcactattaatgaaagtgtaagttattcttcaacggaagatgaaacaaggactcagattttgagcatcaagaaagtcaccccggaggatctcaggcgcaactatgtctgtcatgctcgaaataccaaaggggaagctgagcaggctgccaaggtgaaacagaaagtcataccaccaaggtacacagtagaagtatgtacagaatatccaaatcagatcgttttgtttttatctgtaaatgaaattgatattcgcaagtgtcctcttactccaaataaaatgcacggcgacaccataatttggtacaagaatgacagcaagacccccatatcagcggaccgggactccaggattcatcagcagaatgaacatctttggtttgtacctgccaaggtggaggactcaggatattactattgtatagtaagaaactcaacttactgcctcaaaactaaagtaaccgtaactgtgttagagaatgaccctggcttgtgttacagcacacaggccaccttcccacaggatctccacattgccggggatggaagtcttgtgtgcccttatgtgagttattttaaagatgaaaataatgagttacccgaggtccagtggtataagaactgtaaacctctgcttcttgacaacgtgagcttcttcggagtaaaagataaactgttggtgaggaatgtggctgaagagcacagaggggactatatatgccgtatgtcctatacgttccgggggaagcaatatccggtcacacgagtaatacaatttatcacaatagatgaaaacaagagggacagacctgttatcctgagccctcggaatgagacgatcgaagctgacccaggatcaatgatacaactgatctgcaacgtcacgggccagttctcagaccttgtctactggaagtggaatggatcagaaattgaatggaatgatccatttctagctgaagactatcaatttgtggaacatccttcaaccaaaagaaaatacacactcattacaacacttaacatttcagaagttaaaagccagttttatcgctatccgtttatctgtgttgttaagaacacaaatatttttgagtcggcgcatgtgcagttaatatacccagtccctgacaattcaggtgagcccagagggcccacaatcaagccctgtcctccatgcaaatgcccagcacctaacctcttgggtggaccatccgtcttcatcttccctccaaagatcaaggatgtactcatgatctccctgagccccatagtcacatgtgtggtggtggatgtgagcgaggatgacccagatgtccagatcagctggtttgtgaacaacgtggaagtacacacagctcagacacaaacccatagagaggattacaacagcactctccgggtggtcagtgccctccccatccagcaccaggactggatgagtggcaaggagttcaaatgcaaggtcaacaacaaagacctcccagcgcccatcgagagaaccatctcaaaacccaaagggtcagtaagagctccacaggtatatgtcttgcctccaccagaagaagagatgactaagaaacaggtcactctgacctgcatggtcacagacttcatgcctgaagacatttacgtggagtggaccaacaacgggaaaacagagctaaactacaagaacactgaaccagtcctggactctgatggttcttacttcatgtacagcaagctgagagtggaaaagaagaactgggtggaaagaaatagctactcctgttcagtggtccacgagggtctgcacaatcaccacacgactaagagcttctcccggactccaggtaaataa